European Patent Application EP 4 722 253 A1, published April 8, 2026. Title: CH3 domain variants or bispecific antibodies comprising the same. Applicant: Samsung Biologics. The sequence listing filed with the application follows.

SEQUENCE LISTING (174 sequences)

SEQ ID NO: 1 - protein, 107 aa, synthetic construct
  REGION 1..107: note = Synthetic Sequence
GQPREPQVYTLPPSRDELTKNQVSLTCLVKGFYPSDIAVEWESNGQPENNYKTTPPVLDSDGSFFLYSKLTVDKSRWQQGNVFSCSVMHEALHNHYTQKSLSLSPGK

SEQ ID NO: 2 - protein, 107 aa, synthetic construct; identical to SEQ ID NO: 1
  REGION 1..107: note = Synthetic Sequence

SEQ ID NO: 3 - protein, 567 aa, synthetic construct
  REGION 1..567: note = Synthetic Sequence
EVQLVESGGGLVQPGGSLRLSCAASGFNIKDTYIHWVRQAPGKGLEWVARIYPTNGYTRYADSVKGRFTISADTSKNTAYLQMNSLRAEDTAVYYCSRWGGDGFYAMDYWGQGTLVTVSSASPREPQVYTLPPCREEMTKNQVSLSCAVKGFYPSDIAVEWESNGQPENNYKTTPPVLDSDGSFFLVSKLTVDKSRWQQGNVFSCSVMHEALHNHYTQKSLSLSPGKGGGGSASTKGPSVFPLAPSSKSTSGGTAALGCLVKDYFPEPVTVSWNSGALTSGVHTFPAVLQSSGLYSLSSVVTVPSSSLGTQTYICNVNHKPSNTKVDKKVEPKSSDKTHTCPPCPAPELLGGPSVFLFPPKPKDTLMISRTPEVTCVVVDVSHEDPEVKFNWYVDGVEVHNAKTKPREEQYNSTYRVVSVLTVLHQDWLNGKEYKCKVSNKALPAPIEKTISKAKGQPREPQVYTLPPCTLPPSREEMTKNQVSLSCAVKGFYPSDIAVEWESNGQPENNYKTTPPVLDSDGSFFLVSKLTVDKSRWQQGNVFSCSVMHEALHNHYTQKSLSLSPGK

SEQ ID NO: 4 - protein, 453 aa, synthetic construct
  REGION 1..453: note = Synthetic Sequence
EVQLVESGGGLVQPGGSLRLSCAASGYTFTNYGMNWVRQAPGKGLEWVGWINTYTGEPTYAADFKRRFTFSLDTSKSTAYLQMNSLRAEDTAVYYCAKYPHYYGSSHWYFDVWGQGTLVTVSSASTKGPSVFPLAPSSKSTSGGTAALGCLVKDYFPEPVTVSWNSGALTSGVHTFPAVLQSSGLYSLSSVVTVPSSSLGTQTYICNVNHKPSNTKVDKKVEPKSCDKTHTCPPCPAPELLGGPSVFLFPPKPKDTLMISRTPEVTCVVVDVSHEDPEVKFNWYVDGVEVHNAKTKPREEQYNSTYRVVSVLTVLHQDWLNGKEYKCKVSNKALPAPIEKTISKAKGQPREPQVCTLPPSREEMTKNQVSLWCLVKGFYPSDIAVEWESNGQPENNYKTTPPVLDSDGSFFLYSKLTVDKSRWQQGNVFSCSVMHEALHNHYTQKSLSLSPGK

SEQ ID NO: 5 - protein, 562 aa, synthetic construct
  REGION 1..562: note = Synthetic Sequence
EVQLVESGGGLVQPGGSLRLSCAASGFNIKDTYIHWVRQAPGKGLEWVARIYPTNGYTRYADSVKGRFTISADTSKNTAYLQMNSLRAEDTAVYYCSRWGGDGFYAMDYWGQGTLVTVSSASPREPQVYTLPPCREEMTKNQVSLSCAVKGFYPSDIAVEWESNGQPENNYKTTPPVLDSDGSFFLVSKLTVDKSRWQQGNVFSCSVMHEALHNHYTQKSLSLSPGKGGGGSASTKGPSVFPLAPSSKSTSGGTAALGCLVKDYFPEPVTVSWNSGALTSGVHTFPAVLQSSGLYSLSSVVTVPSSSLGTQTYICNVNHKPSNTKVDKKVEPKSSDKTHTCPPCPAPELLGGPSVFLFPPKPKDTLMISRTPEVTCVVVDVSHEDPEVKFNWYVDGVEVHNAKTKPREEQYNSTYRVVSVLTVLHQDWLNGKEYKCKVSNKALPAPIEKTISKAKGQPREPQVYTLPPCREEMTKNQVSLSCAVKGFYPSDIAVEWESNGQPENNYKTTPPVLDSDGSFFLVSKLTVDKSRWQQGNVFSCSVMHEALHNHYTQDSLSLSPGK

SEQ ID NO: 6 - protein, 453 aa, synthetic construct
  REGION 1..453: note = Synthetic Sequence
EVQLVESGGGLVQPGGSLRLSCAASGYTFTNYGMNWVRQAPGKGLEWVGWINTYTGEPTYAADFKRRFTFSLDTSKSTAYLQMNSLRAEDTAVYYCAKYPHYYGSSHWYFDVWGQGTLVTVSSASTKGPSVFPLAPSSKSTSGGTAALGCLVKDYFPEPVTVSWNSGALTSGVHTFPAVLQSSGLYSLSSVVTVPSSSLGTQTYICNVNHKPSNTKVDKKVEPKSCDKTHTCPPCPAPELLGGPSVFLFPPKPKDTLMISRTPEVTCVVVDVSHEDPEVKFNWYVDGVEVHNAKTKPREEQYNSTYRVVSVLTVLHQDWLNGKEYKCKVSNKALPAPIEKTISKAKGQPREPQVCTLPPSRREMTKNQVSLWCLVKGFYPSDIAVEWESNGQPENNYKTTPPVLDSDGSFFLYSKLTVDKSRWQQGNVFSCSVMHEALHNHYTQKSLSLSPGK

SEQ ID NO: 7 - protein, 562 aa, synthetic construct
  REGION 1..562: note = Synthetic Sequence
EVQLVESGGGLVQPGGSLRLSCAASGFNIKDTYIHWVRQAPGKGLEWVARIYPTNGYTRYADSVKGRFTISADTSKNTAYLQMNSLRAEDTAVYYCSRWGGDGFYAMDYWGQGTLVTVSSASPREPQVYTLPPCREEMTKNQVSLSCAVKGFYPSDIAVEWESNGQPENNYKTTPPVLDSDGSFFLVSKLTVDKSRWQQGNVFSCSVMHEALHNHYTQKSLSLSPGKGGGGSASTKGPSVFPLAPSSKSTSGGTAALGCLVKDYFPEPVTVSWNSGALTSGVHTFPAVLQSSGLYSLSSVVTVPSSSLGTQTYICNVNHKPSNTKVDKKVEPKSSDKTHTCPPCPAPELLGGPSVFLFPPKPKDTLMISRTPEVTCVVVDVSHEDPEVKFNWYVDGVEVHNAKTKPREEQYNSTYRVVSVLTVLHQDWLNGKEYKCKVSNKALPAPIEKTISKAKGQPREPQVYTLPPCREEMTKNQVSLSCAVKGFYPSDIAVEWESNGQPENNYKTTPPVLDSDGSFFLVSVLTVDKSRWQQGNVFSCSVMHEALHNHYTQKSLSLSPGK

SEQ ID NO: 8 - protein, 453 aa, synthetic construct
  REGION 1..453: note = Synthetic Sequence
EVQLVESGGGLVQPGGSLRLSCAASGYTFTNYGMNWVRQAPGKGLEWVGWINTYTGEPTYAADFKRRFTFSLDTSKSTAYLQMNSLRAEDTAVYYCAKYPHYYGSSHWYFDVWGQGTLVTVSSASTKGPSVFPLAPSSKSTSGGTAALGCLVKDYFPEPVTVSWNSGALTSGVHTFPAVLQSSGLYSLSSVVTVPSSSLGTQTYICNVNHKPSNTKVDKKVEPKSCDKTHTCPPCPAPELLGGPSVFLFPPKPKDTLMISRTPEVTCVVVDVSHEDPEVKFNWYVDGVEVHNAKTKPREEQYNSTYRVVSVLTVLHQDWLNGKEYKCKVSNKALPAPIEKTISKAKGQPREPQVCTLPPSREEMTKNQVSLWCLVKGFYPSDIAVEWESNGQPENNYKTTPPVLHSDGSFFLYSKLTVDKSRWQQGNVFSCSVMHEALHNHYTQKSLSLSPGK

SEQ ID NO: 9 - protein, 562 aa, synthetic construct
  REGION 1..562: note = Synthetic Sequence
EVQLVESGGGLVQPGGSLRLSCAASGFNIKDTYIHWVRQAPGKGLEWVARIYPTNGYTRYADSVKGRFTISADTSKNTAYLQMNSLRAEDTAVYYCSRWGGDGFYAMDYWGQGTLVTVSSASPREPQVYTLPPCREEMTKNQVSLSCAVKGFYPSDIAVEWESNGQPENNYKTTPPVLDSDGSFFLVSKLTVDKSRWQQGNVFSCSVMHEALHNHYTQKSLSLSPGKGGGGSASTKGPSVFPLAPSSKSTSGGTAALGCLVKDYFPEPVTVSWNSGALTSGVHTFPAVLQSSGLYSLSSVVTVPSSSLGTQTYICNVNHKPSNTKVDKKVEPKSSDKTHTCPPCPAPELLGGPSVFLFPPKPKDTLMISRTPEVTCVVVDVSHEDPEVKFNWYVDGVEVHNAKTKPREEQYNSTYRVVSVLTVLHQDWLNGKEYKCKVSNKALPAPIEKTISKAKGQPREPQVYTLPPCREEMTKNQVSLSCAVNGFYPSDIAVEWESNGQPENNYKTTPPVLDSDGSFFLVSKLTVDKSRWQQGNVFSCSVMHEALHNHYTQKSLSLSPGK

SEQ ID NO: 10 - protein, 453 aa, synthetic construct
  REGION 1..453: note = Synthetic Sequence
EVQLVESGGGLVQPGGSLRLSCAASGYTFTNYGMNWVRQAPGKGLEWVGWINTYTGEPTYAADFKRRFTFSLDTSKSTAYLQMNSLRAEDTAVYYCAKYPHYYGSSHWYFDVWGQGTLVTVSSASTKGPSVFPLAPSSKSTSGGTAALGCLVKDYFPEPVTVSWNSGALTSGVHTFPAVLQSSGLYSLSSVVTVPSSSLGTQTYICNVNHKPSNTKVDKKVEPKSCDKTHTCPPCPAPELLGGPSVFLFPPKPKDTLMISRTPEVTCVVVDVSHEDPEVKFNWYVDGVEVHNAKTKPREEQYNSTYRVVSVLTVLHQDWLNGKEYKCKVSNKALPAPIEKTISKAKGQPREPQVCTLPPSRERMTKNQVSLWCLVKGFYPSDIAVEWESNGQPENNYKTTPPVLDSDGSFFLYSKLTVDKSRWQQGNVFSCSVMHEALHNHYTQKSLSLSPGK

SEQ ID NO: 11 - protein, 562 aa, synthetic construct
  REGION 1..562: note = Synthetic Sequence
EVQLVESGGGLVQPGGSLRLSCAASGFNIKDTYIHWVRQAPGKGLEWVARIYPTNGYTRYADSVKGRFTISADTSKNTAYLQMNSLRAEDTAVYYCSRWGGDGFYAMDYWGQGTLVTVSSASPREPQVYTLPPCREEMTKNQVSLSCAVKGFYPSDIAVEWESNGQPENNYKTTPPVLDSDGSFFLVSKLTVDKSRWQQGNVFSCSVMHEALHNHYTQKSLSLSPGKGGGGSASTKGPSVFPLAPSSKSTSGGTAALGCLVKDYFPEPVTVSWNSGALTSGVHTFPAVLQSSGLYSLSSVVTVPSSSLGTQTYICNVNHKPSNTKVDKKVEPKSSDKTHTCPPCPAPELLGGPSVFLFPPKPKDTLMISRTPEVTCVVVDVSHEDPEVKFNWYVDGVEVHNAKTKPREEQYNSTYRVVSVLTVLHQDWLNGKEYKCKVSNKALPAPIEKTISKAKGQPREPQVYTLPPCREEMTKNQVSLSCAVKGFYPSDIAVEWESNGQPENNYKTTPPVLDSDGSFFLVSVLTVDKSRWQQGNVFSCSVMHEALHNHYTQDSLSLSPGK

SEQ ID NO: 12 - protein, 453 aa, synthetic construct
  REGION 1..453: note = Synthetic Sequence
EVQLVESGGGLVQPGGSLRLSCAASGYTFTNYGMNWVRQAPGKGLEWVGWINTYTGEPTYAADFKRRFTFSLDTSKSTAYLQMNSLRAEDTAVYYCAKYPHYYGSSHWYFDVWGQGTLVTVSSASTKGPSVFPLAPSSKSTSGGTAALGCLVKDYFPEPVTVSWNSGALTSGVHTFPAVLQSSGLYSLSSVVTVPSSSLGTQTYICNVNHKPSNTKVDKKVEPKSCDKTHTCPPCPAPELLGGPSVFLFPPKPKDTLMISRTPEVTCVVVDVSHEDPEVKFNWYVDGVEVHNAKTKPREEQYNSTYRVVSVLTVLHQDWLNGKEYKCKVSNKALPAPIEKTISKAKGQPREPQVCTLPPSRREMTKNQVSLWCLVKGFYPSDIAVEWESNGQPENNYKTTPPVLHSDGSFFLYSKLTVDKSRWQQGNVFSCSVMHEALHNHYTQKSLSLSPGK

SEQ ID NO: 13 - protein, 562 aa, synthetic construct
  REGION 1..562: note = Synthetic Sequence
EVQLVESGGGLVQPGGSLRLSCAASGFNIKDTYIHWVRQAPGKGLEWVARIYPTNGYTRYADSVKGRFTISADTSKNTAYLQMNSLRAEDTAVYYCSRWGGDGFYAMDYWGQGTLVTVSSASPREPQVYTLPPCREEMTKNQVSLSCAVKGFYPSDIAVEWESNGQPENNYKTTPPVLDSDGSFFLVSKLTVDKSRWQQGNVFSCSVMHEALHNHYTQKSLSLSPGKGGGGSASTKGPSVFPLAPSSKSTSGGTAALGCLVKDYFPEPVTVSWNSGALTSGVHTFPAVLQSSGLYSLSSVVTVPSSSLGTQTYICNVNHKPSNTKVDKKVEPKSSDKTHTCPPCPAPELLGGPSVFLFPPKPKDTLMISRTPEVTCVVVDVSHEDPEVKFNWYVDGVEVHNAKTKPREEQYNSTYRVVSVLTVLHQDWLNGKEYKCKVSNKALPAPIEKTISKAKGQPREPQVYTLPPCREEMTKNQVSLSCAVNGFYPSDIAVEWESNGQPENNYKTTPPVLDSDGSFFLVSKLTVDKSRWQQGNVFSCSVMHEALHNHYTQDSLSLSPGK

SEQ ID NO: 14 - protein, 453 aa, synthetic construct
  REGION 1..453: note = Synthetic Sequence
EVQLVESGGGLVQPGGSLRLSCAASGYTFTNYGMNWVRQAPGKGLEWVGWINTYTGEPTYAADFKRRFTFSLDTSKSTAYLQMNSLRAEDTAVYYCAKYPHYYGSSHWYFDVWGQGTLVTVSSASTKGPSVFPLAPSSKSTSGGTAALGCLVKDYFPEPVTVSWNSGALTSGVHTFPAVLQSSGLYSLSSVVTVPSSSLGTQTYICNVNHKPSNTKVDKKVEPKSCDKTHTCPPCPAPELLGGPSVFLFPPKPKDTLMISRTPEVTCVVVDVSHEDPEVKFNWYVDGVEVHNAKTKPREEQYNSTYRVVSVLTVLHQDWLNGKEYKCKVSNKALPAPIEKTISKAKGQPREPQVCTLPPSRRRMTKNQVSLWCLVKGFYPSDIAVEWESNGQPENNYKTTPPVLDSDGSFFLYSKLTVDKSRWQQGNVFSCSVMHEALHNHYTQKSLSLSPGK

SEQ ID NO: 15 - protein, 562 aa, synthetic construct
  REGION 1..562: note = Synthetic Sequence
EVQLVESGGGLVQPGGSLRLSCAASGFNIKDTYIHWVRQAPGKGLEWVARIYPTNGYTRYADSVKGRFTISADTSKNTAYLQMNSLRAEDTAVYYCSRWGGDGFYAMDYWGQGTLVTVSSASPREPQVYTLPPCREEMTKNQVSLSCAVKGFYPSDIAVEWESNGQPENNYKTTPPVLDSDGSFFLVSKLTVDKSRWQQGNVFSCSVMHEALHNHYTQKSLSLSPGKGGGGSASTKGPSVFPLAPSSKSTSGGTAALGCLVKDYFPEPVTVSWNSGALTSGVHTFPAVLQSSGLYSLSSVVTVPSSSLGTQTYICNVNHKPSNTKVDKKVEPKSSDKTHTCPPCPAPELLGGPSVFLFPPKPKDTLMISRTPEVTCVVVDVSHEDPEVKFNWYVDGVEVHNAKTKPREEQYNSTYRVVSVLTVLHQDWLNGKEYKCKVSNKALPAPIEKTISKAKGQPREPQVYTLPPCREEMTKNQVSLSCAVNGFYPSDIAVEWESNGQPENNYKTTPPVLDSDGSFFLVSVLTVDKSRWQQGNVFSCSVMHEALHNHYTQKSLSLSPGK

SEQ ID NO: 16 - protein, 453 aa, synthetic construct
  REGION 1..453: note = Synthetic Sequence
EVQLVESGGGLVQPGGSLRLSCAASGYTFTNYGMNWVRQAPGKGLEWVGWINTYTGEPTYAADFKRRFTFSLDTSKSTAYLQMNSLRAEDTAVYYCAKYPHYYGSSHWYFDVWGQGTLVTVSSASTKGPSVFPLAPSSKSTSGGTAALGCLVKDYFPEPVTVSWNSGALTSGVHTFPAVLQSSGLYSLSSVVTVPSSSLGTQTYICNVNHKPSNTKVDKKVEPKSCDKTHTCPPCPAPELLGGPSVFLFPPKPKDTLMISRTPEVTCVVVDVSHEDPEVKFNWYVDGVEVHNAKTKPREEQYNSTYRVVSVLTVLHQDWLNGKEYKCKVSNKALPAPIEKTISKAKGQPREPQVCTLPPSRERMTKNQVSLWCLVKGFYPSDIAVEWESNGQPENNYKTTPPVLHSDGSFFLYSKLTVDKSRWQQGNVFSCSVMHEALHNHYTQKSLSLSPGK

SEQ ID NO: 17 - protein, 562 aa, synthetic construct
  REGION 1..562: note = Synthetic Sequence
EVQLVESGGGLVQPGGSLRLSCAASGFNIKDTYIHWVRQAPGKGLEWVARIYPTNGYTRYADSVKGRFTISADTSKNTAYLQMNSLRAEDTAVYYCSRWGGDGFYAMDYWGQGTLVTVSSASPREPQVYTLPPCREEMTKNQVSLSCAVKGFYPSDIAVEWESNGQPENNYKTTPPVLDSDGSFFLVSKLTVDKSRWQQGNVFSCSVMHEALHNHYTQKSLSLSPGKGGGGSASTKGPSVFPLAPSSKSTSGGTAALGCLVKDYFPEPVTVSWNSGALTSGVHTFPAVLQSSGLYSLSSVVTVPSSSLGTQTYICNVNHKPSNTKVDKKVEPKSSDKTHTCPPCPAPELLGGPSVFLFPPKPKDTLMISRTPEVTCVVVDVSHEDPEVKFNWYVDGVEVHNAKTKPREEQYNSTYRVVSVLTVLHQDWLNGKEYKCKVSNKALPAPIEKTISKAKGQPREPQVYTLPPCREEMTKNQVSLSCAVNGFYPSDIAVEWESNGQPENNYKTTPPVLDSDGSFFLVSVLTVDKSRWQQGNVFSCSVMHEALHNHYTQDSLSLSPGK

SEQ ID NO: 18 - protein, 453 aa, synthetic construct
  REGION 1..453: note = Synthetic Sequence
EVQLVESGGGLVQPGGSLRLSCAASGYTFTNYGMNWVRQAPGKGLEWVGWINTYTGEPTYAADFKRRFTFSLDTSKSTAYLQMNSLRAEDTAVYYCAKYPHYYGSSHWYFDVWGQGTLVTVSSASTKGPSVFPLAPSSKSTSGGTAALGCLVKDYFPEPVTVSWNSGALTSGVHTFPAVLQSSGLYSLSSVVTVPSSSLGTQTYICNVNHKPSNTKVDKKVEPKSCDKTHTCPPCPAPELLGGPSVFLFPPKPKDTLMISRTPEVTCVVVDVSHEDPEVKFNWYVDGVEVHNAKTKPREEQYNSTYRVVSVLTVLHQDWLNGKEYKCKVSNKALPAPIEKTISKAKGQPREPQVCTLPPSRRRMTKNQVSLWCLVKGFYPSDIAVEWESNGQPENNYKTTPPVLHSDGSFFLYSKLTVDKSRWQQGNVFSCSVMHEALHNHYTQKSLSLSPGK

SEQ ID NO: 19 - protein, 562 aa, synthetic construct
  REGION 1..562: note = Synthetic Sequence
EVQLVESGGGLVQPGGSLRLSCAASGFNIKDTYIHWVRQAPGKGLEWVARIYPTNGYTRYADSVKGRFTISADTSKNTAYLQMNSLRAEDTAVYYCSRWGGDGFYAMDYWGQGTLVTVSSASPREPQVCTLPPSREEMTKNQVSLSCAVKGFYPSDIAVEWESNGQPENNYKTTPPVLDSDGSFFLVSKLTVDKSRWQQGNVFSCSVMHEALHNHYTQKSLSLSPGKGGGGSASTKGPSVFPLAPSSKSTSGGTAALGCLVKDYFPEPVTVSWNSGALTSGVHTFPAVLQSSGLYSLSSVVTVPSSSLGTQTYICNVNHKPSNTKVDKKVEPKSSDKTHTCPPCPAPELLGGPSVFLFPPKPKDTLMISRTPEVTCVVVDVSHEDPEVKFNWYVDGVEVHNAKTKPREEQYNSTYRVVSVLTVLHQDWLNGKEYKCKVSNKALPAPIEKTISKAKGQPREPQVYTLPPCREEMTKNQVSLSCAVKGFYPSDIAVEWESNGQPENNYKTTPPVLDSDGSFFLVSKLTVDKSRWQQGNVFSCSVMHEALHNHYTQKSLSLSPGK

SEQ ID NO: 20 - protein, 453 aa, synthetic construct; identical to SEQ ID NO: 4
  REGION 1..453: note = Synthetic Sequence

SEQ ID NO: 21 - protein, 562 aa, synthetic construct
  REGION 1..562: note = Synthetic Sequence
EVQLVESGGGLVQPGGSLRLSCAASGFNIKDTYIHWVRQAPGKGLEWVARIYPTNGYTRYADSVKGRFTISADTSKNTAYLQMNSLRAEDTAVYYCSRWGGDGFYAMDYWGQGTLVTVSSASPREPQVCTLPPSREEMTKNQVSLSCAVKGFYPSDIAVEWESNGQPENNYKTTPPVLDSDGSFFLVSKLTVDKSRWQQGNVFSCSVMHEALHNHYTQKSLSLSPGKGGGGSASTKGPSVFPLAPSSKSTSGGTAALGCLVKDYFPEPVTVSWNSGALTSGVHTFPAVLQSSGLYSLSSVVTVPSSSLGTQTYICNVNHKPSNTKVDKKVEPKSSDKTHTCPPCPAPELLGGPSVFLFPPKPKDTLMISRTPEVTCVVVDVSHEDPEVKFNWYVDGVEVHNAKTKPREEQYNSTYRVVSVLTVLHQDWLNGKEYKCKVSNKALPAPIEKTISKAKGQPREPQVYTLPPCREEMTKNQVSLSCAVKGFYPSDIAVEWESNGQPENNYKTTPPVLDSDGSFFLVSKLTVDKSRWQQGNVFSCSVMHEALHNHYTQDSLSLSPGK

SEQ ID NO: 22 - protein, 453 aa, synthetic construct; identical to SEQ ID NO: 6
  REGION 1..453: note = Synthetic Sequence

SEQ ID NO: 23 - protein, 562 aa, synthetic construct
  REGION 1..562: note = Synthetic Sequence
EVQLVESGGGLVQPGGSLRLSCAASGFNIKDTYIHWVRQAPGKGLEWVARIYPTNGYTRYADSVKGRFTISADTSKNTAYLQMNSLRAEDTAVYYCSRWGGDGFYAMDYWGQGTLVTVSSASPREPQVCTLPPSREEMTKNQVSLSCAVKGFYPSDIAVEWESNGQPENNYKTTPPVLDSDGSFFLVSVLTVDKSRWQQGNVFSCSVMHEALHNHYTQKSLSLSPGKGGGGSASTKGPSVFPLAPSSKSTSGGTAALGCLVKDYFPEPVTVSWNSGALTSGVHTFPAVLQSSGLYSLSSVVTVPSSSLGTQTYICNVNHKPSNTKVDKKVEPKSSDKTHTCPPCPAPELLGGPSVFLFPPKPKDTLMISRTPEVTCVVVDVSHEDPEVKFNWYVDGVEVHNAKTKPREEQYNSTYRVVSVLTVLHQDWLNGKEYKCKVSNKALPAPIEKTISKAKGQPREPQVYTLPPCREEMTKNQVSLSCAVKGFYPSDIAVEWESNGQPENNYKTTPPVLDSDGSFFLVSKLTVDKSRWQQGNVFSCSVMHEALHNHYTQDSLSLSPGK

SEQ ID NO: 24 - protein, 453 aa, synthetic construct; identical to SEQ ID NO: 6
  REGION 1..453: note = Synthetic Sequence

SEQ ID NO: 25 - protein, 562 aa, synthetic construct
  REGION 1..562: note = Synthetic Sequence
EVQLVESGGGLVQPGGSLRLSCAASGFNIKDTYIHWVRQAPGKGLEWVARIYPTNGYTRYADSVKGRFTISADTSKNTAYLQMNSLRAEDTAVYYCSRWGGDGFYAMDYWGQGTLVTVSSASPREPQVCTLPPSREEMTKNQVSLSCAVNGFYPSDIAVEWESNGQPENNYKTTPPVLDSDGSFFLVSKLTVDKSRWQQGNVFSCSVMHEALHNHYTQKSLSLSPGKGGGGSASTKGPSVFPLAPSSKSTSGGTAALGCLVKDYFPEPVTVSWNSGALTSGVHTFPAVLQSSGLYSLSSVVTVPSSSLGTQTYICNVNHKPSNTKVDKKVEPKSSDKTHTCPPCPAPELLGGPSVFLFPPKPKDTLMISRTPEVTCVVVDVSHEDPEVKFNWYVDGVEVHNAKTKPREEQYNSTYRVVSVLTVLHQDWLNGKEYKCKVSNKALPAPIEKTISKAKGQPREPQVYTLPPCREEMTKNQVSLSCAVKGFYPSDIAVEWESNGQPENNYKTTPPVLDSDGSFFLVSKLTVDKSRWQQGNVFSCSVMHEALHNHYTQDSLSLSPGK

SEQ ID NO: 26 - protein, 453 aa, synthetic construct; identical to SEQ ID NO: 6
  REGION 1..453: note = Synthetic Sequence

SEQ ID NO: 27 - protein, 562 aa, synthetic construct
  REGION 1..562: note = Synthetic Sequence
EVQLVESGGGLVQPGGSLRLSCAASGFNIKDTYIHWVRQAPGKGLEWVARIYPTNGYTRYADSVKGRFTISADTSKNTAYLQMNSLRAEDTAVYYCSRWGGDGFYAMDYWGQGTLVTVSSASPREPQVYTLPPCREEMTKNQVSLSCAVKGFYPSDIAVEWESNGQPENNYKTTPPVLHSDGSFFLVSKLTVDKSRWQQGNVFSCSVMHEALHNHYTQKSLSLSPGKGGGGSASTKGPSVFPLAPSSKSTSGGTAALGCLVKDYFPEPVTVSWNSGALTSGVHTFPAVLQSSGLYSLSSVVTVPSSSLGTQTYICNVNHKPSNTKVDKKVEPKSSDKTHTCPPCPAPELLGGPSVFLFPPKPKDTLMISRTPEVTCVVVDVSHEDPEVKFNWYVDGVEVHNAKTKPREEQYNSTYRVVSVLTVLHQDWLNGKEYKCKVSNKALPAPIEKTISKAKGQPREPQVYTLPPCREEMTKNQVSLSCAVKGFYPSDIAVEWESNGQPENNYKTTPPVLDSDGSFFLVSKLTVDKSRWQQGNVFSCSVMHEALHNHYTQDSLSLSPGK

SEQ ID NO: 28 - protein, 453 aa, synthetic construct; identical to SEQ ID NO: 6
  REGION 1..453: note = Synthetic Sequence

SEQ ID NO: 29 - protein, 562 aa, synthetic construct
  REGION 1..562: note = Synthetic Sequence
EVQLVESGGGLVQPGGSLRLSCAASGFNIKDTYIHWVRQAPGKGLEWVARIYPTNGYTRYADSVKGRFTISADTSKNTAYLQMNSLRAEDTAVYYCSRWGGDGFYAMDYWGQGTLVTVSSASPREPQVYTLPPCRERMTKNQVSLSCAVKGFYPSDIAVEWESNGQPENNYKTTPPVLDSDGSFFLVSKLTVDKSRWQQGNVFSCSVMHEALHNHYTQKSLSLSPGKGGGGSASTKGPSVFPLAPSSKSTSGGTAALGCLVKDYFPEPVTVSWNSGALTSGVHTFPAVLQSSGLYSLSSVVTVPSSSLGTQTYICNVNHKPSNTKVDKKVEPKSSDKTHTCPPCPAPELLGGPSVFLFPPKPKDTLMISRTPEVTCVVVDVSHEDPEVKFNWYVDGVEVHNAKTKPREEQYNSTYRVVSVLTVLHQDWLNGKEYKCKVSNKALPAPIEKTISKAKGQPREPQVYTLPPCREEMTKNQVSLSCAVKGFYPSDIAVEWESNGQPENNYKTTPPVLDSDGSFFLVSKLTVDKSRWQQGNVFSCSVMHEALHNHYTQDSLSLSPGK

SEQ ID NO: 30 - protein, 453 aa, synthetic construct; identical to SEQ ID NO: 6
  REGION 1..453: note = Synthetic Sequence

SEQ ID NO: 31 - protein, 562 aa, synthetic construct
  REGION 1..562: note = Synthetic Sequence
EVQLVESGGGLVQPGGSLRLSCAASGFNIKDTYIHWVRQAPGKGLEWVARIYPTNGYTRYADSVKGRFTISADTSKNTAYLQMNSLRAEDTAVYYCSRWGGDGFYAMDYWGQGTLVTVSSASPREPQVCTLPPSREEMTKNQVSLSCAVKGFYPSDIAVEWESNGQPENNYKTTPPVLDSDGSFFLVSKLTVDKSRWQQGNVFSCSVMHEALHNHYTQKSLSLSPGKGGGGSASTKGPSVFPLAPSSKSTSGGTAALGCLVKDYFPEPVTVSWNSGALTSGVHTFPAVLQSSGLYSLSSVVTVPSSSLGTQTYICNVNHKPSNTKVDKKVEPKSSDKTHTCPPCPAPELLGGPSVFLFPPKPKDTLMISRTPEVTCVVVDVSHEDPEVKFNWYVDGVEVHNAKTKPREEQYNSTYRVVSVLTVLHQDWLNGKEYKCKVSNKALPAPIEKTISKAKGQPREPQVYTLPPCREEMTKNQVSLSCAVKGFYPSDIAVEWESNGQPENNYKTTPPVLDSDGSFFLVSVLTVDKSRWQQGNVFSCSVMHEALHNHYTQKSLSLSPGK

SEQ ID NO: 32 - protein, 453 aa, synthetic construct; identical to SEQ ID NO: 8
  REGION 1..453: note = Synthetic Sequence

SEQ ID NO: 33 - protein, 562 aa, synthetic construct
  REGION 1..562: note = Synthetic Sequence
EVQLVESGGGLVQPGGSLRLSCAASGFNIKDTYIHWVRQAPGKGLEWVARIYPTNGYTRYADSVKGRFTISADTSKNTAYLQMNSLRAEDTAVYYCSRWGGDGFYAMDYWGQGTLVTVSSASPREPQVCTLPPSREEMTKNQVSLSCAVKGFYPSDIAVEWESNGQPENNYKTTPPVLDSDGSFFLVSKLTVDKSRWQQGNVFSCSVMHEALHNHYTQKSLSLSPGKGGGGSASTKGPSVFPLAPSSKSTSGGTAALGCLVKDYFPEPVTVSWNSGALTSGVHTFPAVLQSSGLYSLSSVVTVPSSSLGTQTYICNVNHKPSNTKVDKKVEPKSSDKTHTCPPCPAPELLGGPSVFLFPPKPKDTLMISRTPEVTCVVVDVSHEDPEVKFNWYVDGVEVHNAKTKPREEQYNSTYRVVSVLTVLHQDWLNGKEYKCKVSNKALPAPIEKTISKAKGQPREPQVYTLPPCREEMTKNQVSLSCAVNGFYPSDIAVEWESNGQPENNYKTTPPVLDSDGSFFLVSKLTVDKSRWQQGNVFSCSVMHEALHNHYTQKSLSLSPGK

SEQ ID NO: 34 - protein, 453 aa, synthetic construct; identical to SEQ ID NO: 10
  REGION 1..453: note = Synthetic Sequence

SEQ ID NO: 35 - protein, 562 aa, synthetic construct
  REGION 1..562: note = Synthetic Sequence
EVQLVESGGGLVQPGGSLRLSCAASGFNIKDTYIHWVRQAPGKGLEWVARIYPTNGYTRYADSVKGRFTISADTSKNTAYLQMNSLRAEDTAVYYCSRWGGDGFYAMDYWGQGTLVTVSSASPREPQVCTLPPSREEMTKNQVSLSCAVKGFYPSDIAVEWESNGQPENNYKTTPPVLDSDGSFFLVSKLTVDKSRWQQGNVFSCSVMHEALHNHYTQKSLSLSPGKGGGGSASTKGPSVFPLAPSSKSTSGGTAALGCLVKDYFPEPVTVSWNSGALTSGVHTFPAVLQSSGLYSLSSVVTVPSSSLGTQTYICNVNHKPSNTKVDKKVEPKSSDKTHTCPPCPAPELLGGPSVFLFPPKPKDTLMISRTPEVTCVVVDVSHEDPEVKFNWYVDGVEVHNAKTKPREEQYNSTYRVVSVLTVLHQDWLNGKEYKCKVSNKALPAPIEKTISKAKGQPREPQVYTLPPCREEMTKNQVSLSCAVKGFYPSDIAVEWESNGQPENNYKTTPPVLDSDGSFFLVSKLTVDKSRWQQGNVFSCSVMHEALHNHYTQNSLSLSPGK

SEQ ID NO: 36 - protein, 453 aa, synthetic construct
  REGION 1..453: note = Synthetic Sequence
EVQLVESGGGLVQPGGSLRLSCAASGYTFTNYGMNWVRQAPGKGLEWVGWINTYTGEPTYAADFKRRFTFSLDTSKSTAYLQMNSLRAEDTAVYYCAKYPHYYGSSHWYFDVWGQGTLVTVSSASTKGPSVFPLAPSSKSTSGGTAALGCLVKDYFPEPVTVSWNSGALTSGVHTFPAVLQSSGLYSLSSVVTVPSSSLGTQTYICNVNHKPSNTKVDKKVEPKSCDKTHTCPPCPAPELLGGPSVFLFPPKPKDTLMISRTPEVTCVVVDVSHEDPEVKFNWYVDGVEVHNAKTKPREEQYNSTYRVVSVLTVLHQDWLNGKEYKCKVSNKALPAPIEKTISKAKGQPREPQVCTLPPSRKEMTKNQVSLWCLVKGFYPSDIAVEWESNGQPENNYKTTPPVLDSDGSFFLYSKLTVDKSRWQQGNVFSCSVMHEALHNHYTQKSLSLSPGK

SEQ ID NO: 37 - protein, 562 aa, synthetic construct
  REGION 1..562: note = Synthetic Sequence
EVQLVESGGGLVQPGGSLRLSCAASGFNIKDTYIHWVRQAPGKGLEWVARIYPTNGYTRYADSVKGRFTISADTSKNTAYLQMNSLRAEDTAVYYCSRWGGDGFYAMDYWGQGTLVTVSSASPREPQVCTLPPSREEMTKNQVSLSCAVKGFYPSDIAVEWESNGQPENNYKTTPPVLDSDGSFFLVSKLTVDKSRWQQGNVFSCSVMHEALHNHYTQKSLSLSPGKGGGGSASTKGPSVFPLAPSSKSTSGGTAALGCLVKDYFPEPVTVSWNSGALTSGVHTFPAVLQSSGLYSLSSVVTVPSSSLGTQTYICNVNHKPSNTKVDKKVEPKSSDKTHTCPPCPAPELLGGPSVFLFPPKPKDTLMISRTPEVTCVVVDVSHEDPEVKFNWYVDGVEVHNAKTKPREEQYNSTYRVVSVLTVLHQDWLNGKEYKCKVSNKALPAPIEKTISKAKGQPREPQVYTLPPCREEMTKNQVSLSCAVKGFYPSDIAVEWESNGQPENNYKTTPPVLDSDGSFFLVSKLTVDKSRWQQGNVFSCSVMHEALHNHYTQQSLSLSPGK

SEQ ID NO: 38 - protein, 453 aa, synthetic construct; identical to SEQ ID NO: 36
  REGION 1..453: note = Synthetic Sequence

SEQ ID NO: 39 - protein, 562 aa, synthetic construct
  REGION 1..562: note = Synthetic Sequence
EVQLVESGGGLVQPGGSLRLSCAASGFNIKDTYIHWVRQAPGKGLEWVARIYPTNGYTRYADSVKGRFTISADTSKNTAYLQMNSLRAEDTAVYYCSRWGGDGFYAMDYWGQGTLVTVSSASPREPQVCTLPPSREEMTKNQVSLSCAVNGFYPSDIAVEWESNGQPENNYKTTPPVLDSDGSFFLVSKLTVDKSRWQQGNVFSCSVMHEALHNHYTQKSLSLSPGKGGGGSASTKGPSVFPLAPSSKSTSGGTAALGCLVKDYFPEPVTVSWNSGALTSGVHTFPAVLQSSGLYSLSSVVTVPSSSLGTQTYICNVNHKPSNTKVDKKVEPKSSDKTHTCPPCPAPELLGGPSVFLFPPKPKDTLMISRTPEVTCVVVDVSHEDPEVKFNWYVDGVEVHNAKTKPREEQYNSTYRVVSVLTVLHQDWLNGKEYKCKVSNKALPAPIEKTISKAKGQPREPQVYTLPPCREEMTKNQVSLSCAVKGFYPSDIAVEWESNGQPENNYKTTPPVLDSDGSFFLVSKLTVDKSRWQQGNVFSCSVMHEALHNHYTQNSLSLSPGK

SEQ ID NO: 40 - protein, 453 aa, synthetic construct; identical to SEQ ID NO: 36
  REGION 1..453: note = Synthetic Sequence

SEQ ID NO: 41 - protein, 562 aa, synthetic construct
  REGION 1..562: note = Synthetic Sequence
EVQLVESGGGLVQPGGSLRLSCAASGFNIKDTYIHWVRQAPGKGLEWVARIYPTNGYTRYADSVKGRFTISADTSKNTAYLQMNSLRAEDTAVYYCSRWGGDGFYAMDYWGQGTLVTVSSASPREPQVCTLPPSREEMTKNQVSLSCAVNGFYPSDIAVEWESNGQPENNYKTTPPVLDSDGSFFLVSKLTVDKSRWQQGNVFSCSVMHEALHNHYTQKSLSLSPGKGGGGSASTKGPSVFPLAPSSKSTSGGTAALGCLVKDYFPEPVTVSWNSGALTSGVHTFPAVLQSSGLYSLSSVVTVPSSSLGTQTYICNVNHKPSNTKVDKKVEPKSSDKTHTCPPCPAPELLGGPSVFLFPPKPKDTLMISRTPEVTCVVVDVSHEDPEVKFNWYVDGVEVHNAKTKPREEQYNSTYRVVSVLTVLHQDWLNGKEYKCKVSNKALPAPIEKTISKAKGQPREPQVYTLPPCREEMTKNQVSLSCAVKGFYPSDIAVEWESNGQPENNYKTTPPVLDSDGSFFLVSKLTVDKSRWQQGNVFSCSVMHEALHNHYTQQSLSLSPGK

SEQ ID NO: 42 - protein, 453 aa, synthetic construct; identical to SEQ ID NO: 36
  REGION 1..453: note = Synthetic Sequence

SEQ ID NO: 43 - protein, 562 aa, synthetic construct
  REGION 1..562: note = Synthetic Sequence
EVQLVESGGGLVQPGGSLRLSCAASGFNIKDTYIHWVRQAPGKGLEWVARIYPTNGYTRYADSVKGRFTISADTSKNTAYLQMNSLRAEDTAVYYCSRWGGDGFYAMDYWGQGTLVTVSSASPREPQVCTLPPSREEMTKNQVSLSCAVKGFYPSDIAVEWESNGQPENNYKTTPPVLDSDGSFFLVSKLTVDKSRWQQGNVFSCSVMHEALHNHYTQDSLSLSPGKGGGGSASTKGPSVFPLAPSSKSTSGGTAALGCLVKDYFPEPVTVSWNSGALTSGVHTFPAVLQSSGLYSLSSVVTVPSSSLGTQTYICNVNHKPSNTKVDKKVEPKSSDKTHTCPPCPAPELLGGPSVFLFPPKPKDTLMISRTPEVTCVVVDVSHEDPEVKFNWYVDGVEVHNAKTKPREEQYNSTYRVVSVLTVLHQDWLNGKEYKCKVSNKALPAPIEKTISKAKGQPREPQVYTLPPCREEMTKNQVSLSCAVKGFYPSDIAVEWESNGQPENNYKTTPPVLDSDGSFFLVSVLTVDKSRWQQGNVFSCSVMHEALHNHYTQKSLSLSPGK

SEQ ID NO: 44 - protein, 453 aa, synthetic construct; identical to SEQ ID NO: 8
  REGION 1..453: note = Synthetic Sequence

SEQ ID NO: 45 - protein, 562 aa, synthetic construct
  REGION 1..562: note = Synthetic Sequence
EVQLVESGGGLVQPGGSLRLSCAASGFNIKDTYIHWVRQAPGKGLEWVARIYPTNGYTRYADSVKGRFTISADTSKNTAYLQMNSLRAEDTAVYYCSRWGGDGFYAMDYWGQGTLVTVSSASPREPQVCTLPPSREEMTKNQVSLSCAVKGFYPSDIAVEWESNGQPENNYKTTPPVLDSDGSFFLVSVLTVDKSRWQQGNVFSCSVMHEALHNHYTQKSLSLSPGKGGGGSASTKGPSVFPLAPSSKSTSGGTAALGCLVKDYFPEPVTVSWNSGALTSGVHTFPAVLQSSGLYSLSSVVTVPSSSLGTQTYICNVNHKPSNTKVDKKVEPKSSDKTHTCPPCPAPELLGGPSVFLFPPKPKDTLMISRTPEVTCVVVDVSHEDPEVKFNWYVDGVEVHNAKTKPREEQYNSTYRVVSVLTVLHQDWLNGKEYKCKVSNKALPAPIEKTISKAKGQPREPQVYTLPPCREEMTKNQVSLSCAVKGFYPSDIAVEWESNGQPENNYKTTPPVLDSDGSFFLVSVLTVDKSRWQQGNVFSCSVMHEALHNHYTQKSLSLSPGK

SEQ ID NO: 46 - protein, 453 aa, synthetic construct; identical to SEQ ID NO: 8
  REGION 1..453: note = Synthetic Sequence

SEQ ID NO: 47 - protein, 562 aa, synthetic construct; identical to SEQ ID NO: 35
  REGION 1..562: note = Synthetic Sequence

SEQ ID NO: 48 - protein, 453 aa, synthetic construct; identical to SEQ ID NO: 6
  REGION 1..453: note = Synthetic Sequence

SEQ ID NO: 49 - protein, 562 aa, synthetic construct; identical to SEQ ID NO: 37
  REGION 1..562: note = Synthetic Sequence

SEQ ID NO: 50 - protein, 453 aa, synthetic construct; identical to SEQ ID NO: 6
  REGION 1..453: note = Synthetic Sequence

SEQ ID NO: 51 - protein, 562 aa, synthetic construct; identical to SEQ ID NO: 39
  REGION 1..562: note = Synthetic Sequence

SEQ ID NO: 52 - protein, 453 aa, synthetic construct; identical to SEQ ID NO: 6
  REGION 1..453: note = Synthetic Sequence

SEQ ID NO: 53 - protein, 562 aa, synthetic construct; identical to SEQ ID NO: 41
  REGION 1..562: note = Synthetic Sequence

SEQ ID NO: 54 - protein, 453 aa, synthetic construct; identical to SEQ ID NO: 6
  REGION 1..453: note = Synthetic Sequence

SEQ ID NO: 55 - protein, 562 aa, synthetic construct
  REGION 1..562: note = Synthetic Sequence
EVQLVESGGGLVQPGGSLRLSCAASGFNIKDTYIHWVRQAPGKGLEWVARIYPTNGYTRYADSVKGRFTISADTSKNTAYLQMNSLRAEDTAVYYCSRWGGDGFYAMDYWGQGTLVTVSSASPREPQVCTLPPSREEMTKNQVSLSCAVNGFYPSDIAVEWESNGQPENNYKTTPPVLDSDGSFFLVSKLTVDKSRWQQGNVFSCSVMHEALHNHYTQKSLSLSPGKGGGGSASTKGPSVFPLAPSSKSTSGGTAALGCLVKDYFPEPVTVSWNSGALTSGVHTFPAVLQSSGLYSLSSVVTVPSSSLGTQTYICNVNHKPSNTKVDKKVEPKSSDKTHTCPPCPAPELLGGPSVFLFPPKPKDTLMISRTPEVTCVVVDVSHEDPEVKFNWYVDGVEVHNAKTKPREEQYNSTYRVVSVLTVLHQDWLNGKEYKCKVSNKALPAPIEKTISKAKGQPREPQVYTLPPCREEMTKNQVSLSCAVKGFYPSDIAVEWESNGQPENNYKTTPPVLDSDGSFFLVSVLTVDKSRWQQGNVFSCSVMHEALHNHYTQKSLSLSPGK

SEQ ID NO: 56 - protein, 453 aa, synthetic construct; identical to SEQ ID NO: 8
  REGION 1..453: note = Synthetic Sequence

SEQ ID NO: 57 - protein, 562 aa, synthetic construct; identical to SEQ ID NO: 31
  REGION 1..562: note = Synthetic Sequence

SEQ ID NO: 58 - protein, 453 aa, synthetic construct
  REGION 1..453: note = Synthetic Sequence
EVQLVESGGGLVQPGGSLRLSCAASGYTFTNYGMNWVRQAPGKGLEWVGWINTYTGEPTYAADFKRRFTFSLDTSKSTAYLQMNSLRAEDTAVYYCAKYPHYYGSSHWYFDVWGQGTLVTVSSASTKGPSVFPLAPSSKSTSGGTAALGCLVKDYFPEPVTVSWNSGALTSGVHTFPAVLQSSGLYSLSSVVTVPSSSLGTQTYICNVNHKPSNTKVDKKVEPKSCDKTHTCPPCPAPELLGGPSVFLFPPKPKDTLMISRTPEVTCVVVDVSHEDPEVKFNWYVDGVEVHNAKTKPREEQYNSTYRVVSVLTVLHQDWLNGKEYKCKVSNKALPAPIEKTISKAKGQPREPQVCTLPPSREEMTKNQVSLWCLVKGFYPSDIAVEWESNGQPENNYKTTPPVLFSDGSFFLYSKLTVDKSRWQQGNVFSCSVMHEALHNHYTQKSLSLSPGK

SEQ ID NO: 59 - protein, 562 aa, synthetic construct
  REGION 1..562: note = Synthetic Sequence
EVQLVESGGGLVQPGGSLRLSCAASGFNIKDTYIHWVRQAPGKGLEWVARIYPTNGYTRYADSVKGRFTISADTSKNTAYLQMNSLRAEDTAVYYCSRWGGDGFYAMDYWGQGTLVTVSSASPREPQVCTLPPSREEMTKNQVSLSCAVKGFYPSDIAVEWESNGQPENNYKTTPPVLDSDGSFFLVSKLTVDKSRWQQGNVFSCSVMHEALHNHYTQKSLSLSPGKGGGGSASTKGPSVFPLAPSSKSTSGGTAALGCLVKDYFPEPVTVSWNSGALTSGVHTFPAVLQSSGLYSLSSVVTVPSSSLGTQTYICNVNHKPSNTKVDKKVEPKSSDKTHTCPPCPAPELLGGPSVFLFPPKPKDTLMISRTPEVTCVVVDVSHEDPEVKFNWYVDGVEVHNAKTKPREEQYNSTYRVVSVLTVLHQDWLNGKEYKCKVSNKALPAPIEKTISKAKGQPREPQVYTLPPCREEMTKNQVSLSCAVKGFYPSDIAVEWESNGQPENNYKTTPPVLDSDGSFFLVSTLTVDKSRWQQGNVFSCSVMHEALHNHYTQKSLSLSPGK

SEQ ID NO: 60 - protein, 453 aa, synthetic construct; identical to SEQ ID NO: 58
  REGION 1..453: note = Synthetic Sequence

SEQ ID NO: 61 - protein, 562 aa, synthetic construct; identical to SEQ ID NO: 43
  REGION 1..562: note = Synthetic Sequence

SEQ ID NO: 62 - protein, 453 aa, synthetic construct; identical to SEQ ID NO: 58
  REGION 1..453: note = Synthetic Sequence

SEQ ID NO: 63 - protein, 562 aa, synthetic construct; identical to SEQ ID NO: 43
  REGION 1..562: note = Synthetic Sequence

SEQ ID NO: 64 - protein, 453 aa, synthetic construct; identical to SEQ ID NO: 58
  REGION 1..453: note = Synthetic Sequence

SEQ ID NO: 65 - protein, 562 aa, synthetic construct; identical to SEQ ID NO: 45
  REGION 1..562: note = Synthetic Sequence

SEQ ID NO: 66 - protein, 453 aa, synthetic construct; identical to SEQ ID NO: 58
  REGION 1..453: note = Synthetic Sequence

SEQ ID NO: 67 - protein, 562 aa, synthetic construct
  REGION 1..562: note = Synthetic Sequence
EVQLVESGGGLVQPGGSLRLSCAASGFNIKDTYIHWVRQAPGKGLEWVARIYPTNGYTRYADSVKGRFTISADTSKNTAYLQMNSLRAEDTAVYYCSRWGGDGFYAMDYWGQGTLVTVSSASPREPQVCTLPPSREEMTKNQVSLSCAVKGFYPSDIAVEWESNGQPENNYKTTPPVLDSDGSFFLVSKLTVDKSRWQQGNVFSCSVMHEALHNHYTQKSLSLSPGKGGGGSASTKGPSVFPLAPSSKSTSGGTAALGCLVKDYFPEPVTVSWNSGALTSGVHTFPAVLQSSGLYSLSSVVTVPSSSLGTQTYICNVNHKPSNTKVDKKVEPKSSDKTHTCPPCPAPELLGGPSVFLFPPKPKDTLMISRTPEVTCVVVDVSHEDPEVKFNWYVDGVEVHNAKTKPREEQYNSTYRVVSVLTVLHQDWLNGKEYKCKVSNKALPAPIEKTISKAKGQPREPQVYTLPPCREEMTKNQVSLSCAVKGFYPSDIAVEWESNGQPENNYKTTPPVLFSDGSFFLVSKLTVDKSRWQQGNVFSCSVMHEALHNHYTQKSLSLSPGK

SEQ ID NO: 68 - protein, 453 aa, synthetic construct
  REGION 1..453: note = Synthetic Sequence
EVQLVESGGGLVQPGGSLRLSCAASGYTFTNYGMNWVRQAPGKGLEWVGWINTYTGEPTYAADFKRRFTFSLDTSKSTAYLQMNSLRAEDTAVYYCAKYPHYYGSSHWYFDVWGQGTLVTVSSASTKGPSVFPLAPSSKSTSGGTAALGCLVKDYFPEPVTVSWNSGALTSGVHTFPAVLQSSGLYSLSSVVTVPSSSLGTQTYICNVNHKPSNTKVDKKVEPKSCDKTHTCPPCPAPELLGGPSVFLFPPKPKDTLMISRTPEVTCVVVDVSHEDPEVKFNWYVDGVEVHNAKTKPREEQYNSTYRVVSVLTVLHQDWLNGKEYKCKVSNKALPAPIEKTISKAKGQPREPQVCTLPPSREEMTKNQVSLWCLVKGFYPSDIAVEWESNGQPENNYKTTPPVLDSDGSFFLYSVLTVDKSRWQQGNVFSCSVMHEALHNHYTQKSLSLSPGK

SEQ ID NO: 69 - protein, 562 aa, synthetic construct; identical to SEQ ID NO: 67
  REGION 1..562: note = Synthetic Sequence

SEQ ID NO: 70 - protein, 453 aa, synthetic construct
  REGION 1..453: note = Synthetic Sequence
EVQLVESGGGLVQPGGSLRLSCAASGYTFTNYGMNWVRQAPGKGLEWVGWINTYTGEPTYAADFKRRFTFSLDTSKSTAYLQMNSLRAEDTAVYYCAKYPHYYGSSHWYFDVWGQGTLVTVSSASTKGPSVFPLAPSSKSTSGGTAALGCLVKDYFPEPVTVSWNSGALTSGVHTFPAVLQSSGLYSLSSVVTVPSSSLGTQTYICNVNHKPSNTKVDKKVEPKSCDKTHTCPPCPAPELLGGPSVFLFPPKPKDTLMISRTPEVTCVVVDVSHEDPEVKFNWYVDGVEVHNAKTKPREEQYNSTYRVVSVLTVLHQDWLNGKEYKCKVSNKALPAPIEKTISKAKGQPREPQVCTLPPSREEMTKNQVSLWCLVKGFYPSDIAVEWESNGQPENNYKTTPPVLDSDGSFFLYSTLTVDKSRWQQGNVFSCSVMHEALHNHYTQKSLSLSPGK

SEQ ID NO: 71 - protein, 562 aa, synthetic construct; identical to SEQ ID NO: 67
  REGION 1..562: note = Synthetic Sequence

SEQ ID NO: 72 - protein, 453 aa, synthetic construct
  REGION 1..453: note = Synthetic Sequence
EVQLVESGGGLVQPGGSLRLSCAASGYTFTNYGMNWVRQAPGKGLEWVGWINTYTGEPTYAADFKRRFTFSLDTSKSTAYLQMNSLRAEDTAVYYCAKYPHYYGSSHWYFDVWGQGTLVTVSSASTKGPSVFPLAPSSKSTSGGTAALGCLVKDYFPEPVTVSWNSGALTSGVHTFPAVLQSSGLYSLSSVVTVPSSSLGTQTYICNVNHKPSNTKVDKKVEPKSCDKTHTCPPCPAPELLGGPSVFLFPPKPKDTLMISRTPEVTCVVVDVSHEDPEVKFNWYVDGVEVHNAKTKPREEQYNSTYRVVSVLTVLHQDWLNGKEYKCKVSNKALPAPIEKTISKAKGQPREPQVCTLPPSREEMTKNQVSLWCLVKGFYPSDIAVEWESNGQPENNYKTTPPVLDSDGSFFLYSSLTVDKSRWQQGNVFSCSVMHEALHNHYTQKSLSLSPGK

SEQ ID NO: 73 - protein, 562 aa, synthetic construct
  REGION 1..562: note = Synthetic Sequence
EVQLVESGGGLVQPGGSLRLSCAASGFNIKDTYIHWVRQAPGKGLEWVARIYPTNGYTRYADSVKGRFTISADTSKNTAYLQMNSLRAEDTAVYYCSRWGGDGFYAMDYWGQGTLVTVSSASPREPQVCTLPPSREEMTKNQVSLSCAVKGFYPSDIAVEWESNGQPENNYKTTPPVLDSDGSFFLVSKLTVDKSRWQQGNVFSCSVMHEALHNHYTQKSLSLSPGKGGGGSASTKGPSVFPLAPSSKSTSGGTAALGCLVKDYFPEPVTVSWNSGALTSGVHTFPAVLQSSGLYSLSSVVTVPSSSLGTQTYICNVNHKPSNTKVDKKVEPKSSDKTHTCPPCPAPELLGGPSVFLFPPKPKDTLMISRTPEVTCVVVDVSHEDPEVKFNWYVDGVEVHNAKTKPREEQYNSTYRVVSVLTVLHQDWLNGKEYKCKVSNKALPAPIEKTISKAKGQPREPQVYTLPPCREEMTKNQVSLSCAVKGFYPSDIAVEWESNGQPENNYKTTPPVLYSDGSFFLVSKLTVDKSRWQQGNVFSCSVMHEALHNHYTQKSLSLSPGK

SEQ ID NO: 74 - protein, 453 aa, synthetic construct; identical to SEQ ID NO: 68
  REGION 1..453: note = Synthetic Sequence

SEQ ID NO: 75 - protein, 562 aa, synthetic construct; identical to SEQ ID NO: 73
  REGION 1..562: note = Synthetic Sequence

SEQ ID NO: 76 - protein, 453 aa, synthetic construct; identical to SEQ ID NO: 70
  REGION 1..453: note = Synthetic Sequence

SEQ ID NO: 77 - protein, 562 aa, synthetic construct; identical to SEQ ID NO: 73
  REGION 1..562: note = Synthetic Sequence

SEQ ID NO: 78 - protein, 453 aa, synthetic construct; identical to SEQ ID NO: 72
  REGION 1..453: note = Synthetic Sequence

SEQ ID NO: 79 - protein, 562 aa, synthetic construct
  REGION 1..562: note = Synthetic Sequence
EVQLVESGGGLVQPGGSLRLSCAASGFNIKDTYIHWVRQAPGKGLEWVARIYPTNGYTRYADSVKGRFTISADTSKNTAYLQMNSLRAEDTAVYYCSRWGGDGFYAMDYWGQGTLVTVSSASPREPQVCTLPPSREEMTKNQVSLSCAVKGFYPSDIAVEWESNGQPENNYKTTPPVLDSDGSFFLVSKLTVDKSRWQQGNVFSCSVMHEALHNHYTQKSLSLSPGKGGGGSASTKGPSVFPLAPSSKSTSGGTAALGCLVKDYFPEPVTVSWNSGALTSGVHTFPAVLQSSGLYSLSSVVTVPSSSLGTQTYICNVNHKPSNTKVDKKVEPKSSDKTHTCPPCPAPELLGGPSVFLFPPKPKDTLMISRTPEVTCVVVDVSHEDPEVKFNWYVDGVEVHNAKTKPREEQYNSTYRVVSVLTVLHQDWLNGKEYKCKVSNKALPAPIEKTISKAKGQPREPQVYTLPPCREEMTKNQVSLSCAVKGFYPSDIAVEWESNGQPENNYKTTPPVLHSDGSFFLVSKLTVDKSRWQQGNVFSCSVMHEALHNHYTQKSLSLSPGK

SEQ ID NO: 80 - protein, 453 aa, synthetic construct; identical to SEQ ID NO: 68
  REGION 1..453: note = Synthetic Sequence

SEQ ID NO: 81 - protein, 562 aa, synthetic construct; identical to SEQ ID NO: 79
  REGION 1..562: note = Synthetic Sequence

SEQ ID NO: 82 - protein, 453 aa, synthetic construct; identical to SEQ ID NO: 70
  REGION 1..453: note = Synthetic Sequence

SEQ ID NO: 83 - protein, 562 aa, synthetic construct; identical to SEQ ID NO: 79
  REGION 1..562: note = Synthetic Sequence

SEQ ID NO: 84 - protein, 453 aa, synthetic construct; identical to SEQ ID NO: 72
  REGION 1..453: note = Synthetic Sequence

SEQ ID NO: 85 - protein, 562 aa, synthetic construct
  REGION 1..562: note = Synthetic Sequence
EVQLVESGGGLVQPGGSLRLSCAASGFNIKDTYIHWVRQAPGKGLEWVARIYPTNGYTRYADSVKGRFTISADTSKNTAYLQMNSLRAEDTAVYYCSRWGGDGFYAMDYWGQGTLVTVSSASPREPQVCTLPPSREEMTKNQVSLSCAVKGFYPSDIAVEWESNGQPENNYKTTPPVLDSDGSFFLVSKLTVDKSRWQQGNVFSCSVMHEALHNHYTQKSLSLSPGKGGGGSASTKGPSVFPLAPSSKSTSGGTAALGCLVKDYFPEPVTVSWNSGALTSGVHTFPAVLQSSGLYSLSSVVTVPSSSLGTQTYICNVNHKPSNTKVDKKVEPKSSDKTHTCPPCPAPELLGGPSVFLFPPKPKDTLMISRTPEVTCVVVDVSHEDPEVKFNWYVDGVEVHNAKTKPREEQYNSTYRVVSVLTVLHQDWLNGKEYKCKVSNKALPAPIEKTISKAKGQPREPQVYTLPPCREEMTKNQVSLSCAVKGFYPSDIAVEWESNGQPENNYKTTPPVLWSDGSFFLVSKLTVDKSRWQQGNVFSCSVMHEALHNHYTQKSLSLSPGK

SEQ ID NO: 86 - protein, 453 aa, synthetic construct
  REGION 1..453: note = Synthetic Sequence
EVQLVESGGGLVQPGGSLRLSCAASGYTFTNYGMNWVRQAPGKGLEWVGWINTYTGEPTYAADFKRRFTFSLDTSKSTAYLQMNSLRAEDTAVYYCAKYPHYYGSSHWYFDVWGQGTLVTVSSASTKGPSVFPLAPSSKSTSGGTAALGCLVKDYFPEPVTVSWNSGALTSGVHTFPAVLQSSGLYSLSSVVTVPSSSLGTQTYICNVNHKPSNTKVDKKVEPKSCDKTHTCPPCPAPELLGGPSVFLFPPKPKDTLMISRTPEVTCVVVDVSHEDPEVKFNWYVDGVEVHNAKTKPREEQYNSTYRVVSVLTVLHQDWLNGKEYKCKVSNKALPAPIEKTISKAKGQPREPQVCTLPPSREEMTKNQVSLWCLVKGFYPSDIAVEWESNGQPENNYKTTPPVLDSDGSFFLYSALTVDKSRWQQGNVFSCSVMHEALHNHYTQKSLSLSPGK

SEQ ID NO: 87 - protein, 562 aa, synthetic construct
  REGION 1..562: note = Synthetic Sequence
EVQLVESGGGLVQPGGSLRLSCAASGFNIKDTYIHWVRQAPGKGLEWVARIYPTNGYTRYADSVKGRFTISADTSKNTAYLQMNSLRAEDTAVYYCSRWGGDGFYAMDYWGQGTLVTVSSASPREPQVYTLPPCREEMTKNQVSLSCAVKGFYPSDIAVEWESNGQPENNYKTTPPVLDSDGSFFLVSKLTVDKSRWQQGNVFSCSVMHEALHNHYTQKSLSLSPGKGGGGSASTKGPSVFPLAPSSKSTSGGTAALGCLVKDYFPEPVTVSWNSGALTSGVHTFPAVLQSSGLYSLSSVVTVPSSSLGTQTYICNVNHKPSNTKVDKKVEPKSSDKTHTCPPCPAPELLGGPSVFLFPPKPKDTLMISRTPEVTCVVVDVSHEDPEVKFNWYVDGVEVHNAKTKPREEQYNSTYRVVSVLTVLHQDWLNGKEYKCKVSNKALPAPIEKTISKAKGQPREPQVCTLPPSREEMTKNQVSLSCAVKGFYPSDIAVEWESNGQPENNYKTTPPVLFSDGSFFLVSKLTVDKSRWQQGNVFSCSVMHEALHNHYTQKSLSLSPGK

SEQ ID NO: 88 - protein, 453 aa, synthetic construct
  REGION 1..453: note = Synthetic Sequence
EVQLVESGGGLVQPGGSLRLSCAASGYTFTNYGMNWVRQAPGKGLEWVGWINTYTGEPTYAADFKRRFTFSLDTSKSTAYLQMNSLRAEDTAVYYCAKYPHYYGSSHWYFDVWGQGTLVTVSSASTKGPSVFPLAPSSKSTSGGTAALGCLVKDYFPEPVTVSWNSGALTSGVHTFPAVLQSSGLYSLSSVVTVPSSSLGTQTYICNVNHKPSNTKVDKKVEPKSCDKTHTCPPCPAPELLGGPSVFLFPPKPKDTLMISRTPEVTCVVVDVSHEDPEVKFNWYVDGVEVHNAKTKPREEQYNSTYRVVSVLTVLHQDWLNGKEYKCKVSNKALPAPIEKTISKAKGQPREPQVYTLPPCREEMTKNQVSLWCLVKGFYPSDIAVEWESNGQPENNYKTTPPVLDSDGSFFLYSVLTVDKSRWQQGNVFSCSVMHEALHNHYTQKSLSLSPGK

SEQ ID NO: 89 - protein, 326 aa, synthetic construct
  REGION 1..326: note = Synthetic Sequence
DIQMTQSPSSLSASVGDRVTITCRASQDVNTAVAWYQQKPGKAPKLLIYSASFLYSGVPSRFSGSRSGTDFTLTISSLQPEDFATYYCQQHYTTPPTFGQGTKVEIKRTPREPQVCTLPPSREEMTKNQVSLWCLVKGFYPSDIAVEWESNGQPENNYKTTPPVLDSDGSFFLYSKLTVDKSRWQQGNVFSCSVMHEALHNHYTQKSLSLSPGKGGGGSRTVAAPSVFIFPPSDEQLKSGTASVVCLLNNFYPREAKVQWKVDNALQSGNSQESVTEQDSKDSTYSLSSTLTLSKADYEKHKVYACEVTHQGLSSPVTKSFNRGES

SEQ ID NO: 90 - protein, 214 aa, synthetic construct
  REGION 1..214: note = Synthetic Sequence
DIQMTQSPSSLSASVGDRVTITCSASQDISNYLNWYQQKPGKAPKVLIYFTSSLHSGVPSRFSGSGSGTDFTLTISSLQPEDFATYYCQQYSTVPWTFGQGTKVEIKRTVAAPSVFIFPPSDEQLKSGTASVVCLLNNFYPREAKVQWKVDNALQSGNSQESVTEQDSKDSTYSLSSTLTLSKADYEKHKVYACEVTHQGLSSPVTKSFNRGEC

SEQ ID NO: 91 - protein, 326 aa, synthetic construct; identical to SEQ ID NO: 89
  REGION 1..326: note = Synthetic Sequence

SEQ ID NO: 92 - protein, 214 aa, synthetic construct; identical to SEQ ID NO: 90
  REGION 1..214: note = Synthetic Sequence

SEQ ID NO: 93 - protein, 326 aa, synthetic construct; identical to SEQ ID NO: 89
  REGION 1..326: note = Synthetic Sequence

SEQ ID NO: 94 - protein, 214 aa, synthetic construct; identical to SEQ ID NO: 90
  REGION 1..214: note = Synthetic Sequence

SEQ ID NO: 95 - protein, 326 aa, synthetic construct; identical to SEQ ID NO: 89
  REGION 1..326: note = Synthetic Sequence

SEQ ID NO: 96 - protein, 214 aa, synthetic construct; identical to SEQ ID NO: 90
  REGION 1..214: note = Synthetic Sequence

SEQ ID NO: 97 - protein, 326 aa, synthetic construct; identical to SEQ ID NO: 89
  REGION 1..326: note = Synthetic Sequence

SEQ ID NO: 98 - protein, 214 aa, synthetic construct; identical to SEQ ID NO: 90
  REGION 1..214: note = Synthetic Sequence

SEQ ID NO: 99 - protein, 326 aa, synthetic construct; identical to SEQ ID NO: 89
  REGION 1..326: note = Synthetic Sequence

SEQ ID NO: 100 - protein, 214 aa, synthetic construct; identical to SEQ ID NO: 90
  REGION 1..214: note = Synthetic Sequence

SEQ ID NO: 101 - protein, 326 aa, synthetic construct; identical to SEQ ID NO: 89
  REGION 1..326: note = Synthetic Sequence

SEQ ID NO: 102 - protein, 214 aa, synthetic construct; identical to SEQ ID NO: 90
  REGION 1..214: note = Synthetic Sequence

SEQ ID NO: 103 - protein, 326 aa, synthetic construct; identical to SEQ ID NO: 89
  REGION 1..326: note = Synthetic Sequence

SEQ ID NO: 104 - protein, 214 aa, synthetic construct; identical to SEQ ID NO: 90
  REGION 1..214: note = Synthetic Sequence

SEQ ID NO: 105 - protein, 326 aa, synthetic construct
  REGION 1..326: note = Synthetic Sequence
DIQMTQSPSSLSASVGDRVTITCRASQDVNTAVAWYQQKPGKAPKLLIYSASFLYSGVPSRFSGSRSGTDFTLTISSLQPEDFATYYCQQHYTTPPTFGQGTKVEIKRTPREPQVYTLPPCREEMTKNQVSLWCLVKGFYPSDIAVEWESNGQPENNYKTTPPVLDSDGSFFLYSKLTVDKSRWQQGNVFSCSVMHEALHNHYTQKSLSLSPGKGGGGSRTVAAPSVFIFPPSDEQLKSGTASVVCLLNNFYPREAKVQWKVDNALQSGNSQESVTEQDSKDSTYSLSSTLTLSKADYEKHKVYACEVTHQGLSSPVTKSFNRGES

SEQ ID NO: 106 - protein, 214 aa, synthetic construct; identical to SEQ ID NO: 90
  REGION 1..214: note = Synthetic Sequence

SEQ ID NO: 107 - protein, 326 aa, synthetic construct; identical to SEQ ID NO: 105
  REGION 1..326: note = Synthetic Sequence

SEQ ID NO: 108 - protein, 214 aa, synthetic construct; identical to SEQ ID NO: 90
  REGION 1..214: note = Synthetic Sequence

SEQ ID NO: 109 - protein, 326 aa, synthetic construct
  REGION 1..326: note = Synthetic Sequence
DIQMTQSPSSLSASVGDRVTITCRASQDVNTAVAWYQQKPGKAPKLLIYSASFLYSGVPSRFSGSRSGTDFTLTISSLQPEDFATYYCQQHYTTPPTFGQGTKVEIKRTPREPQVYTLPPCREEMTKNQVSLWCLVKGFYPSDIAVEWESNGQPENNYKTTPPVLHSDGSFFLYSKLTVDKSRWQQGNVFSCSVMHEALHNHYTQKSLSLSPGKGGGGSRTVAAPSVFIFPPSDEQLKSGTASVVCLLNNFYPREAKVQWKVDNALQSGNSQESVTEQDSKDSTYSLSSTLTLSKADYEKHKVYACEVTHQGLSSPVTKSFNRGES

SEQ ID NO: 110 - protein, 214 aa, synthetic construct; identical to SEQ ID NO: 90
  REGION 1..214: note = Synthetic Sequence

SEQ ID NO: 111 - protein, 326 aa, synthetic construct
  REGION 1..326: note = Synthetic Sequence
DIQMTQSPSSLSASVGDRVTITCRASQDVNTAVAWYQQKPGKAPKLLIYSASFLYSGVPSRFSGSRSGTDFTLTISSLQPEDFATYYCQQHYTTPPTFGQGTKVEIKRTPREPQVYTLPPCRERMTKNQVSLWCLVKGFYPSDIAVEWESNGQPENNYKTTPPVLDSDGSFFLYSKLTVDKSRWQQGNVFSCSVMHEALHNHYTQKSLSLSPGKGGGGSRTVAAPSVFIFPPSDEQLKSGTASVVCLLNNFYPREAKVQWKVDNALQSGNSQESVTEQDSKDSTYSLSSTLTLSKADYEKHKVYACEVTHQGLSSPVTKSFNRGES

SEQ ID NO: 112 - protein, 214 aa, synthetic construct; identical to SEQ ID NO: 90
  REGION 1..214: note = Synthetic Sequence

SEQ ID NO: 113 - protein, 326 aa, synthetic construct
  REGION 1..326: note = Synthetic Sequence
DIQMTQSPSSLSASVGDRVTITCRASQDVNTAVAWYQQKPGKAPKLLIYSASFLYSGVPSRFSGSRSGTDFTLTISSLQPEDFATYYCQQHYTTPPTFGQGTKVEIKRTPREPQVCTLPPSREEMTKNQVSLWCLVKGFYPSDIAVEWESNGQPENNYKTTPPVLDSDGSFFLYSVLTVDKSRWQQGNVFSCSVMHEALHNHYTQKSLSLSPGKGGGGSRTVAAPSVFIFPPSDEQLKSGTASVVCLLNNFYPREAKVQWKVDNALQSGNSQESVTEQDSKDSTYSLSSTLTLSKADYEKHKVYACEVTHQGLSSPVTKSFNRGES

SEQ ID NO: 114 - protein, 214 aa, synthetic construct; identical to SEQ ID NO: 90
  REGION 1..214: note = Synthetic Sequence

SEQ ID NO: 115 - protein, 326 aa, synthetic construct
  REGION 1..326: note = Synthetic Sequence
DIQMTQSPSSLSASVGDRVTITCRASQDVNTAVAWYQQKPGKAPKLLIYSASFLYSGVPSRFSGSRSGTDFTLTISSLQPEDFATYYCQQHYTTPPTFGQGTKVEIKRTPREPQVCTLPPSREEMTKNQVSLWCLVNGFYPSDIAVEWESNGQPENNYKTTPPVLDSDGSFFLYSKLTVDKSRWQQGNVFSCSVMHEALHNHYTQKSLSLSPGKGGGGSRTVAAPSVFIFPPSDEQLKSGTASVVCLLNNFYPREAKVQWKVDNALQSGNSQESVTEQDSKDSTYSLSSTLTLSKADYEKHKVYACEVTHQGLSSPVTKSFNRGES

SEQ ID NO: 116 - protein, 214 aa, synthetic construct; identical to SEQ ID NO: 90
  REGION 1..214: note = Synthetic Sequence

SEQ ID NO: 117 - protein, 326 aa, synthetic construct; identical to SEQ ID NO: 105
  REGION 1..326: note = Synthetic Sequence

SEQ ID NO: 118 - protein, 214 aa, synthetic construct; identical to SEQ ID NO: 90
  REGION 1..214: note = Synthetic Sequence

SEQ ID NO: 119 - protein, 326 aa, synthetic construct; identical to SEQ ID NO: 105
  REGION 1..326: note = Synthetic Sequence

SEQ ID NO: 120 - protein, 214 aa, synthetic construct; identical to SEQ ID NO: 90
  REGION 1..214: note = Synthetic Sequence

SEQ ID NO: 121 - protein, 326 aa, synthetic construct; identical to SEQ ID NO: 105
  REGION 1..326: note = Synthetic Sequence

SEQ ID NO: 122 - protein, 214 aa, synthetic construct; identical to SEQ ID NO: 90
  REGION 1..214: note = Synthetic Sequence

SEQ ID NO: 123 - protein, 326 aa, synthetic construct; identical to SEQ ID NO: 105
  REGION 1..326: note = Synthetic Sequence

SEQ ID NO: 124 - protein, 214 aa, synthetic construct; identical to SEQ ID NO: 90
  REGION 1..214: note = Synthetic Sequence

SEQ ID NO: 125 - protein, 326 aa, synthetic construct; identical to SEQ ID NO: 111
  REGION 1..326: note = Synthetic Sequence

SEQ ID NO: 126 - protein, 214 aa, synthetic construct; identical to SEQ ID NO: 90
  REGION 1..214: note = Synthetic Sequence

SEQ ID NO: 127 - protein, 326 aa, synthetic construct; identical to SEQ ID NO: 111
  REGION 1..326: note = Synthetic Sequence

SEQ ID NO: 128 - protein, 214 aa, synthetic construct; identical to SEQ ID NO: 90
  REGION 1..214: note = Synthetic Sequence

SEQ ID NO: 129 - protein, 326 aa, synthetic construct
  REGION 1..326: note = Synthetic Sequence
DIQMTQSPSSLSASVGDRVTITCRASQDVNTAVAWYQQKPGKAPKLLIYSASFLYSGVPSRFSGSRSGTDFTLTISSLQPEDFATYYCQQHYTTPPTFGQGTKVEIKRTPREPQVYTLPPCRREMTKNQVSLWCLVKGFYPSDIAVEWESNGQPENNYKTTPPVLDSDGSFFLYSKLTVDKSRWQQGNVFSCSVMHEALHNHYTQKSLSLSPGKGGGGSRTVAAPSVFIFPPSDEQLKSGTASVVCLLNNFYPREAKVQWKVDNALQSGNSQESVTEQDSKDSTYSLSSTLTLSKADYEKHKVYACEVTHQGLSSPVTKSFNRGES

SEQ ID NO: 130 - protein, 214 aa, synthetic construct; identical to SEQ ID NO: 90
  REGION 1..214: note = Synthetic Sequence

SEQ ID NO: 131 - protein, 326 aa, synthetic construct; identical to SEQ ID NO: 109
  REGION 1..326: note = Synthetic Sequence

SEQ ID NO: 132 - protein, 214 aa, synthetic construct; identical to SEQ ID NO: 90
  REGION 1..214: note = Synthetic Sequence

SEQ ID NO: 133 - protein, 326 aa, synthetic construct; identical to SEQ ID NO: 105
  REGION 1..326: note = Synthetic Sequence

SEQ ID NO: 134 - protein, 214 aa, synthetic construct; identical to SEQ ID NO: 90
  REGION 1..214: note = Synthetic Sequence

SEQ ID NO: 135 - protein, 326 aa, synthetic construct; identical to SEQ ID NO: 105
  REGION 1..326: note = Synthetic Sequence

SEQ ID NO: 136 - protein, 214 aa, synthetic construct; identical to SEQ ID NO: 90
  REGION 1..214: note = Synthetic Sequence

SEQ ID NO: 137 - protein, 326 aa, synthetic construct; identical to SEQ ID NO: 111
  REGION 1..326: note = Synthetic Sequence

SEQ ID NO: 138 - protein, 214 aa, synthetic construct; identical to SEQ ID NO: 90
  REGION 1..214: note = Synthetic Sequence

SEQ ID NO: 139 - protein, 326 aa, synthetic construct; identical to SEQ ID NO: 111
  REGION 1..326: note = Synthetic Sequence

SEQ ID NO: 140 - protein, 214 aa, synthetic construct; identical to SEQ ID NO: 90
  REGION 1..214: note = Synthetic Sequence

SEQ ID NO: 141 - protein, 326 aa, synthetic construct; identical to SEQ ID NO: 105
  REGION 1..326: note = Synthetic Sequence

SEQ ID NO: 142 - protein, 214 aa, synthetic construct; identical to SEQ ID NO: 90
  REGION 1..214: note = Synthetic Sequence

SEQ ID NO: 143 - protein, 326 aa, synthetic construct; identical to SEQ ID NO: 105
  REGION 1..326: note = Synthetic Sequence

SEQ ID NO: 144 - protein, 214 aa, synthetic construct; identical to SEQ ID NO: 90
  REGION 1..214: note = Synthetic Sequence

SEQ ID NO: 145 - protein, 326 aa, synthetic construct; identical to SEQ ID NO: 105
  REGION 1..326: note = Synthetic Sequence

SEQ ID NO: 146 - protein, 214 aa, synthetic construct; identical to SEQ ID NO: 90
  REGION 1..214: note = Synthetic Sequence

SEQ ID NO: 147 - protein, 326 aa, synthetic construct; identical to SEQ ID NO: 105
  REGION 1..326: note = Synthetic Sequence

SEQ ID NO: 148 - protein, 214 aa, synthetic construct; identical to SEQ ID NO: 90
  REGION 1..214: note = Synthetic Sequence

SEQ ID NO: 149 - protein, 326 aa, synthetic construct; identical to SEQ ID NO: 129
  REGION 1..326: note = Synthetic Sequence

SEQ ID NO: 150 - protein, 214 aa, synthetic construct; identical to SEQ ID NO: 90
  REGION 1..214: note = Synthetic Sequence

SEQ ID NO: 151 - protein, 326 aa, synthetic construct; identical to SEQ ID NO: 109
  REGION 1..326: note = Synthetic Sequence

SEQ ID NO: 152 - protein, 214 aa, synthetic construct; identical to SEQ ID NO: 90
  REGION 1..214: note = Synthetic Sequence

SEQ ID NO: 153 - protein, 326 aa, synthetic construct; identical to SEQ ID NO: 105
  REGION 1..326: note = Synthetic Sequence

SEQ ID NO: 154 - protein, 214 aa, synthetic construct; identical to SEQ ID NO: 90
  REGION 1..214: note = Synthetic Sequence

SEQ ID NO: 155 - protein, 326 aa, synthetic construct; identical to SEQ ID NO: 105
  REGION 1..326: note = Synthetic Sequence

SEQ ID NO: 156 - protein, 214 aa, synthetic construct; identical to SEQ ID NO: 90
  REGION 1..214: note = Synthetic Sequence

SEQ ID NO: 157 - protein, 326 aa, synthetic construct; identical to SEQ ID NO: 105
  REGION 1..326: note = Synthetic Sequence

SEQ ID NO: 158 - protein, 214 aa, synthetic construct; identical to SEQ ID NO: 90
  REGION 1..214: note = Synthetic Sequence

SEQ ID NO: 159 - protein, 326 aa, synthetic construct; identical to SEQ ID NO: 105
  REGION 1..326: note = Synthetic Sequence

SEQ ID NO: 160 - protein, 214 aa, synthetic construct; identical to SEQ ID NO: 90
  REGION 1..214: note = Synthetic Sequence

SEQ ID NO: 161 - protein, 326 aa, synthetic construct; identical to SEQ ID NO: 105
  REGION 1..326: note = Synthetic Sequence

SEQ ID NO: 162 - protein, 214 aa, synthetic construct; identical to SEQ ID NO: 90
  REGION 1..214: note = Synthetic Sequence

SEQ ID NO: 163 - protein, 326 aa, synthetic construct; identical to SEQ ID NO: 105
  REGION 1..326: note = Synthetic Sequence

SEQ ID NO: 164 - protein, 214 aa, synthetic construct; identical to SEQ ID NO: 90
  REGION 1..214: note = Synthetic Sequence

SEQ ID NO: 165 - protein, 326 aa, synthetic construct; identical to SEQ ID NO: 105
  REGION 1..326: note = Synthetic Sequence

SEQ ID NO: 166 - protein, 214 aa, synthetic construct; identical to SEQ ID NO: 90
  REGION 1..214: note = Synthetic Sequence

SEQ ID NO: 167 - protein, 326 aa, synthetic construct; identical to SEQ ID NO: 105
  REGION 1..326: note = Synthetic Sequence

SEQ ID NO: 168 - protein, 214 aa, synthetic construct; identical to SEQ ID NO: 90
  REGION 1..214: note = Synthetic Sequence

SEQ ID NO: 169 - protein, 326 aa, synthetic construct; identical to SEQ ID NO: 105
  REGION 1..326: note = Synthetic Sequence

SEQ ID NO: 170 - protein, 214 aa, synthetic construct; identical to SEQ ID NO: 90
  REGION 1..214: note = Synthetic Sequence

SEQ ID NO: 171 - protein, 326 aa, synthetic construct; identical to SEQ ID NO: 105
  REGION 1..326: note = Synthetic Sequence

SEQ ID NO: 172 - protein, 214 aa, synthetic construct; identical to SEQ ID NO: 90
  REGION 1..214: note = Synthetic Sequence

SEQ ID NO: 173 - protein, 326 aa, synthetic construct; identical to SEQ ID NO: 89
  REGION 1..326: note = Synthetic Sequence

SEQ ID NO: 174 - protein, 214 aa, synthetic construct; identical to SEQ ID NO: 90
  REGION 1..214: note = Synthetic Sequence